European Patent Application EP 4 600 260 A1, published August 13, 2025. Title: keratin YK93-4, AND preparation method thereof, pharmaceutical composition thereof and use thereof. Applicant: Institute of Materia Medica Chinese Academy Of Medical Sciences. The sequence listing filed with the application follows.

SEQUENCE LISTING (2 sequences)

SEQ ID NO: 1 - protein, 486 aa, Manis pentadactyla
MTCGSYCAGGAFSCASACGPKPGRCCITAAPYSGVSCYRGITGAFGSRSVCGAFRSGSCGRSFGYRAGGVSGPTPPCITSVSVNESLLTPLNLEIDPNAQCVKQEEKEQIKCLNSRFAAFIDKVRFLEQQNKLLETKWQFYQNRQCCESNLEPLFNGYIETLRREAECAEADSGRLASELNHVQEVLEGYKKKYEEEVSLRATAENEFVALKKDVDCAYIRKSDLEANVEALTQEIDFLRRLYEEEIRVLQSHISDTSVIVKMDNSRDLNMDSIVAEIKAQYDDIASRSRAEAESWYRTKCEEIKATVIRHGETLRRTKEEINELNRMIQRLTAEVENAKCQNSKLEAAVTQAEQQGEAALSDARCKLAGLEAALQKAKQDMACLLKEYQEVMNSKLGLDIEIATYRRLLEGEEQRLCEGVGSVNVCVSSSRGGVVCGDLCASGAAPAVSTRVCSAPCSGNMVVGTAAPCAPCTGVSACSVGCKKC

SEQ ID NO: 2 - DNA, 1458 bp, Manis pentadactyla
  source 1..1458: mol_type = genomic DNA
atgacctgtggcagctattgtgccggcggcgcattttcttgtgcaagcgcctgtggtccgaaaccgggccgttgctgtattaccgcagccccgtatagtggtgtgagctgctatcgtggcattaccggcgcctttggtagccgcagcgtttgtggtgcctttcgcagtggtagctgtggccgcagttttggctatcgtgccggtggcgttagcggtccgacccctccttgcattaccagtgtgagcgtgaatgaaagcctgctgaccccgctgaatctggaaattgatccgaatgcacagtgtgtgaaacaggaagaaaaagaacagattaagtgtctgaatagtcgttttgccgcctttattgataaagttcgttttctggaacagcagaataagctgctggaaaccaaatggcagttttatcagaatcgtcagtgctgtgaaagtaatctggaaccgctgtttaatggttatattgaaaccctgcgtcgtgaagccgaatgtgcagaagccgatagtggtcgtctggccagcgaactgaatcatgtgcaggaagttctggaaggctataaaaagaaatatgaagaagaggttagcctgcgtgcaaccgccgaaaatgaatttgtggcactgaaaaaagatgtggattgcgcctatattcgtaaaagtgatctggaagcaaatgtggaagcactgacccaggaaattgattttctgcgtcgcctgtatgaagaagaaattcgcgtgctgcagagtcatattagtgataccagtgtgattgtgaaaatggataatagccgtgatctgaatatggatagtattgttgcagaaattaaggcccagtatgatgatattgcaagccgcagccgtgcagaagcagaaagctggtatcgtaccaaatgcgaagaaattaaggcgaccgtgattcgtcatggcgaaaccctgcgccgcaccaaagaagaaattaatgaactgaatcgcatgattcagcgtctgaccgcagaagtggaaaatgcaaaatgccagaatagtaaactggaagccgcagttacccaggcagaacagcagggcgaagccgcactgagtgatgcacgttgcaaactggccggtctggaagccgccctgcagaaagcaaaacaggatatggcatgtctgctgaaagaatatcaggaagtgatgaatagtaagctgggtctggatattgaaattgcaacctatcgtcgcctgctggaaggtgaagaacagcgcctgtgtgaaggcgtgggtagtgtgaatgtgtgtgttagtagtagtcgtggtggtgttgtgtgcggtgacctgtgcgcaagcggtgccgcccctgcagttagtacccgtgtttgtagtgccccgtgcagcggtaatatggtggttggcaccgccgccccgtgcgcaccttgtacaggcgttagcgcctgcagcgttggttgcaaaaaatgt